European Patent Specification EP 4 486 916 B1, published September 2, 2026. Title: DOUBLE-STRANDED SPLINT ADAPTORS AND METHODS OF USE. Applicant: Element Biosciences, Inc. Application US. The sequence listing filed with the application follows.

SEQUENCE LISTING (212 sequences)

SEQ ID NO: 1-192 - skipped (192 entries)

SEQ ID NO: 193 - DNA, 20 bp, synthetic construct
  misc_feature 1..20: note = first region of the first splint strand (320)
  source 1..20: mol_type = other DNA
tcggtggtcgccgtatcatt

SEQ ID NO: 194 - DNA, 24 bp, synthetic construct
  misc_feature 1..24: note = first region of the first splint strant (320)
  source 1..24: mol_type = other DNA
aatgatacggcgaccaccgagatc

SEQ ID NO: 195 - DNA, 21 bp, synthetic construct
  misc_feature 1..21: note = second region (330)
  source 1..21: mol_type = other DNA
caagcagaagacggcatacga

SEQ ID NO: 196 - DNA, 24 bp, synthetic construct
  misc_feature 1..24: note = second region (330)
  source 1..24: mol_type = other DNA
caagcagaagacggcatacgagat

SEQ ID NO: 197 - DNA, 25 bp, synthetic construct
  misc_feature 1..25: note = internal region (310) sub-region
  source 1..25: mol_type = other DNA
accctgaaagtacgtgcattacatg

SEQ ID NO: 198 - DNA, 23 bp, synthetic construct
  misc_feature 1..23: note = internal region (310) sub-region
  source 1..23: mol_type = other DNA
gatcaggtgaggctgcgacgact

SEQ ID NO: 199 - DNA, 89 bp, synthetic construct
  misc_feature 1..89: note = full length first splint strand (300)
  source 1..89: mol_type = other DNA
tcggtggtcgccgtatcattaccctgaaagtacgtgcattacatggatcaggtgaggctgcgacgactcaagcagaagacggcatacga

SEQ ID NO: 200 - DNA, 25 bp, synthetic construct
  misc_feature 1..25: note = first sub-region of the second splint strand (400)
  source 1..25: mol_type = other DNA
catgtaatgcacgtactttcagggt

SEQ ID NO: 201 - DNA, 23 bp, synthetic construct
  misc_feature 1..23: note = second sub-region of the second splint strand (400)
  source 1..23: mol_type = other DNA
agtcgtcgcagcctcacctgatc

SEQ ID NO: 202 - DNA, 48 bp, synthetic construct
  misc_feature 1..48: note = first and second sub-region
  source 1..48: mol_type = other DNA
agtcgtcgcagcctcacctgatccatgtaatgcacgtactttcagggt

SEQ ID NO: 203 - DNA, 20 bp, synthetic construct
  misc_feature 1..20: note = left universal binding sequence
  source 1..20: mol_type = other DNA
aatgatacggcgaccaccga

SEQ ID NO: 204 - DNA, 33 bp, synthetic construct
  misc_feature 1..33: note = left universal binding sequence
  source 1..33: mol_type = other DNA
acactctttccctacacgacgctcttccgatct

SEQ ID NO: 205 - DNA, 34 bp, synthetic construct
  misc_feature 1..34: note = right universal binding sequence
  source 1..34: mol_type = other DNA
agatcggaagagcacacgtctgaactccagtcac

SEQ ID NO: 206 - DNA, 21 bp, synthetic construct
  misc_feature 1..21: note = right universal binding sequence
  source 1..21: mol_type = other DNA
tcgtatgccgtcttctgcttg

SEQ ID NO: 207 - DNA, 33 bp, synthetic construct
  misc_feature 1..33: note = left universal binding sequence
  source 1..33: mol_type = other DNA
tcgtcggcagcgtcagatgtgtataagagacag

SEQ ID NO: 208 - DNA, 35 bp, synthetic construct
  misc_feature 1..35: note = left universal binding sequence
  source 1..35: mol_type = other DNA
cgtgctggattggctcaccagacaccttccgacat

SEQ ID NO: 209 - DNA, 34 bp, synthetic construct
  misc_feature 1..34: note = right universal binding sequence
  source 1..34: mol_type = other DNA
ctgtctcttatacacatctccgagcccacgagac

SEQ ID NO: 210 - DNA, 35 bp, synthetic construct
  misc_feature 1..35: note = right universal binding sequence
  source 1..35: mol_type = other DNA
atgtcggaaggtgtgcaggctaccgcttgtcaact

SEQ ID NO: 211 - DNA, 19 bp, synthetic construct
  misc_feature 1..19: note = Tn5 transposon-end sequence
  source 1..19: mol_type = other DNA
agatgtgtataagagacag

SEQ ID NO: 212 - DNA, 19 bp, synthetic construct
  misc_feature 1..19: note = Tn5 transposon-end sequence
  source 1..19: mol_type = other DNA
ctgtctcttatacacatct